European Patent Application EP 4 116 327 A1, published January 11, 2023. Title: HUMAN PD-L1 ANTIBODIES AND METHODS OF USE THEREFOR. Applicant: Board of Regents, The University of Texas System. Application EP18866472.6. The sequence listing filed with the application follows.

SEQUENCE LISTING (51 sequences)

SEQ ID NO: 1 - protein, 290 aa, Homo sapiens
MRIFAVFIFMTYWHLLNAFTVTVPKDLYVVEYGSNMTIECKFPVEKQLDLAALIVYWEMEDKNIIQFVHGEEDLKVQHSSYRQRARLLKDQLSLGNAALQITDVKLQDAGVYRCMISYGGADYKRITVKVNAPYNKINQRILVVDPVTSEHELTCQAEGYPKAEVIWTSSDHQVLSGKTTTTNSKREEKLFNVTSTLRINTTTNEIFYCTFRRLDPEENHTAELVIPELPLAHPPNERTHLVILGAILLCLGVALTFIFRLRKGRMMDVKKCGIQDTNSKKQSDTHLEET

SEQ ID NO: 2 - DNA, 366 bp, Homo sapiens
caggtgcagctggtgcagtctggggctgaggtgaagaagcctggggcctcagtgaaggtttcctgcaaggcatctggatacaccttcaccagctactatatgcactgggtgcgacaggcccctggacaagggcttgagtggatgggaataatcaaccctagtggtggtagcacaagctacgcacagaagttccagggcagagtcaccatgaccagggacacgtccacgagcacagtctacatggagctgagcagcctgagatctgaggacacggcggtgtactactgcgccagagatcctttgatgagcggaacacgatggctattcgacatatggggtcagggtacaatggtcaccgtctcctca

SEQ ID NO: 3 - DNA, 321 bp, Homo sapiens
gacatccagatgacccagtctccatcttccgtgtctgcatctgtaggagacagagtcaccatcacttgtcgggcgagtcagggtattagcagctggttagcctggtatcagcagaaaccagggaaagcccctaagctcctgatctatgctgcatccagtttgcaaagtggggtcccatcaaggttcagcggcagtggatctgggacagatttcactctcaccatcagcagcctgcagcctgaagattttgcaacttattactgtcagcaggtacaccacttccctcctacttttggcggagggaccaaggttgagatcaaa

SEQ ID NO: 4 - DNA, 357 bp, Homo sapiens
gaggtgcagctggtggagtctgggggaggcttggtccagcctggggggtccctgagactctcctgtgcagcctctggattcacctttagtagctattggatgagctgggtccgccaggctccagggaagggactggagtgggtggccaacataaagtcagatggaagtgagaaatactatgtggactctgtgaagggccgattcaccatctccagagacaacgccaagaactcactgtatctgcaaatgaacagcctgagagccgaggacacggcggtgtactactgcgccagagtgacatactgggccgactacatggacgtatggggcaagggtacaactgtcaccgtctcctca

SEQ ID NO: 5 - DNA, 321 bp, Homo sapiens
gacatccagatgacccagtctccttccaccctgtctgcatctgtaggagacagagtcaccatcacttgccgggccagtcagagtattagtagctggttggcctggtatcagcagaaaccagggaaagcccctaagctcctgatctataaagcctccagtttggaaagtggggtcccatcaaggttcagcggcagtggatctgggacagaattcactctcaccatcagcagcctgcagcctgatgattttgcaacttattactgccagcagtccggaagtctccctcctacttttggcggagggaccaaggttgagatcaaa

SEQ ID NO: 6 - DNA, 366 bp, Homo sapiens
caggtgcagctggtgcagtctggggctgaggtgaagaagcctgggtcctcggtgaaggtctcctgcaaggcttctggaggcaccttcaggttgtatgctatcagctgggtgcgacaggcccctggacaagggcttgagtggatgggaagtatcatccctggttttggttctgcaaactacgcacagaagttccagggcagagtcacgattaccgcggacgaatccacgagcacagcctacatggagctgagcagcctgagatctgaggacacggcggtgtactactgcgccagagatggtggcggaggaacaagcgcctatagcttcgacccatggggacagggtacattggtcaccgtctcctca

SEQ ID NO: 7 - DNA, 321 bp, Homo sapiens
gaaattgtgttgacacagtctccagccaccctgtctttgtctccaggggaaagagccaccctctcctgcagggccagtcagagtgttagcagctacttagcctggtaccaacagaaacctggccaggctcccaggctcctcatctatgatgcatccaacagggccactggcatcccagccaggttcagtggcagtgggtctgggacagacttcactctcaccatcagcagcctagagcctgaagattttgcagtttattactgtcagcagtccatcaatttcccttacacttttggcggagggaccaaggttgagatcaaa

SEQ ID NO: 8 - DNA, 351 bp, Homo sapiens
caggtgcagctggtgcagtctggggctgaggtgaagaagcctggggcctcagtgaaggtctcctgcaaggcttctggatacaccttcaccggtgtgtatatgcactgggtgcgacaggcccctggacaagggcttgagtggatgggagggatatttcctatcgggggtacagcaaactacgcacagaagttccagggcagagtcacgattaccgcggacgaatccacgagcacagcctacatggagctgagcagcctgagatctgaggacacggcggtgtactactgcgccagagacagaacatccggggccctatactggggacagggtacattggtcaccgtctcctca

SEQ ID NO: 9 - DNA, 321 bp, Homo sapiens
gacatccagatgacccagtctccttccaccctgtctgcatctgtaggagacagagtcaccatcacttgccgggccagtcagagtattagtagctggttggcctggtatcagcagaaaccagggaaagcccctaagctcctgatctataaagcctccagtttggaaagtggggtcccatcaaggttcagcggcagtggatctgggacagaattcactctcaccatcagcagcctgcagcctgatgattttgcaacttattactgccagcagtacaatagcttctcttggacttttggcggagggaccaaggttgagatcaaa

SEQ ID NO: 10 - DNA, 363 bp, Homo sapiens
caggtgcagctgcaggagtcgggcccaggactggtgaagccttcacagaccctgtccctcacctgtactgtctctggtggctccatcgtgagtggtggtttgtactggagctggatccgccagcacccagggaagggcctggagtggattgggtacatctattacgcgggggtgacctactacaacccgtccctcaagagtcgagttaccatatcagtagacacgtctaagaaccagttctccctgaagctgagttctgtgaccgccgcagacacggcggtgtactactgcgccagaggaccaagaatgggattggcaggaatggacgtatggggccagggaacaactgtcaccgtctcctca

SEQ ID NO: 11 - DNA, 321 bp, Homo sapiens
gacatccagatgacccagtctccatcttccgtgtctgcatctgtaggagacagagtcaccatcacttgtcgggcgagtcagggtattagcagctggttagcctggtatcagcagaaaccagggaaagcccctaagctcctgatctatgctgcatccagtttgcaaagtggggtcccatcaaggttcagcggcagtggatctgggacagatttcactctcaccatcagcagcctgcagcctgaagattttgcaacttactattgtcaacaggctaacagtttccctatcacctttggcggagggaccaaggttgagatcaaa

SEQ ID NO: 12 - protein, 122 aa, Homo sapiens
QVQLVQSGAEVKKPGASVKVSCKASGYTFTSYYMHWVRQAPGQGLEWMGIINPSGGSTSYAQKFQGRVTMTRDTSTSTVYMELSSLRSEDTAVYYCARDPLMSGTRWLFDIWGQGTMVTVSS

SEQ ID NO: 13 - protein, 107 aa, Homo sapiens
DIQMTQSPSSVSASVGDRVTITCRASQGISSWLAWYQQKPGKAPKLLIYAASSLQSGVPSRFSGSGSGTDFTLTISSLQPEDFATYYCQQVHHFPPTFGGGTKVEIK

SEQ ID NO: 14 - protein, 119 aa, Homo sapiens
EVQLVESGGGLVQPGGSLRLSCAASGFTFSSYWMSWVRQAPGKGLEWVANIKSDGSEKYYVDSVKGRFTISRDNAKNSLYLQMNSLRAEDTAVYYCARVTYWADYMDVWGKGTTVTVSS

SEQ ID NO: 15 - protein, 107 aa, Homo sapiens
DIQMTQSPSTLSASVGDRVTITCRASQSISSWLAWYQQKPGKAPKLLIYKASSLESGVPSRFSGSGSGTEFTLTISSLQPDDFATYYCQQSGSLPPTFGGGTKVEIK

SEQ ID NO: 16 - protein, 122 aa, Homo sapiens
QVQLVQSGAEVKKPGSSVKVSCKASGGTFRLYAISWVRQAPGQGLEWMGSIIPGFGSANYAQKFQGRVTITADESTSTAYMELSSLRSEDTAVYYCARDGGGGTSAYSFDPWGQGTLVTVSS

SEQ ID NO: 17 - protein, 107 aa, Homo sapiens
EIVLTQSPATLSLSPGERATLSCRASQSVSSYLAWYQQKPGQAPRLLIYDASNRATGIPARFSGSGSGTDFTLTISSLEPEDFAVYYCQQSINFPYTFGGGTKVEIK

SEQ ID NO: 18 - protein, 117 aa, Homo sapiens
QVQLVQSGAEVKKPGASVKVSCKASGYTFTGVYMHWVRQAPGQGLEWMGGIFPIGGTANYAQKFQGRVTITADESTSTAYMELSSLRSEDTAVYYCARDRTSGALYWGQGTLVTVSS

SEQ ID NO: 19 - protein, 107 aa, Homo sapiens
DIQMTQSPSTLSASVGDRVTITCRASQSISSWLAWYQQKPGKAPKLLIYKASSLESGVPSRFSGSGSGTEFTLTISSLQPDDFATYYCQQYNSFSWTFGGGTKVEIK

SEQ ID NO: 20 - protein, 121 aa, Homo sapiens
QVQLQESGPGLVKPSQTLSLTCTVSGGSIVSGGLYWSWIRQHPGKGLEWIGYIYYAGVTYYNPSLKSRVTISVDTSKNQFSLKLSSVTAADTAVYYCARGPRMGLAGMDVWGQGTTVTVSS

SEQ ID NO: 21 - protein, 107 aa, Homo sapiens
DIQMTQSPSSVSASVGDRVTITCRASQGISSWLAWYQQKPGKAPKLLIYAASSLQSGVPSRFSGSGSGTDFTLTISSLQPEDFATYYCQQANSFPITFGGGTKVEIK

SEQ ID NO: 22 - protein, 9 aa, Homo sapiens
YTFTSYYMH

SEQ ID NO: 23 - protein, 17 aa, Homo sapiens
IINPSGGSTSYAQKFQG

SEQ ID NO: 24 - protein, 15 aa, Homo sapiens
ARDPLMSGTRWLFDI

SEQ ID NO: 25 - protein, 9 aa, Homo sapiens
FTFSSYWMS

SEQ ID NO: 26 - protein, 17 aa, Homo sapiens
NIKSDGSEKYYVDSVKG

SEQ ID NO: 27 - protein, 12 aa, Homo sapiens
ARVTYWADYMDV

SEQ ID NO: 28 - protein, 9 aa, Homo sapiens
GTFRLYAIS

SEQ ID NO: 29 - protein, 17 aa, Homo sapiens
SIIPGFGSANYAQKFQG

SEQ ID NO: 30 - protein, 15 aa, Homo sapiens
ARDGGGGTSAYSFDP

SEQ ID NO: 31 - protein, 9 aa, Homo sapiens
YTFTGVYMH

SEQ ID NO: 32 - protein, 17 aa, Homo sapiens
GIFPIGGTANYAQKFQG

SEQ ID NO: 33 - protein, 10 aa, Homo sapiens
ARDRTSGALY

SEQ ID NO: 34 - protein, 11 aa, Homo sapiens
GSIVSGGLYWS

SEQ ID NO: 35 - protein, 16 aa, Homo sapiens
YIYYAGVTYYNPSLKS

SEQ ID NO: 36 - protein, 13 aa, Homo sapiens
ARGPRMGLAGMDV

SEQ ID NO: 37 - protein, 11 aa, Homo sapiens
RASQGISSWLA

SEQ ID NO: 38 - protein, 7 aa, Homo sapiens
AASSLQS

SEQ ID NO: 39 - protein, 9 aa, Homo sapiens
QQVHHFPPT

SEQ ID NO: 40 - protein, 11 aa, Homo sapiens
RASQSISSWLA

SEQ ID NO: 41 - protein, 7 aa, Homo sapiens
KASSLES

SEQ ID NO: 42 - protein, 9 aa, Homo sapiens
QQSGSLPPT

SEQ ID NO: 43 - protein, 11 aa, Homo sapiens
RASQSVSSYLA

SEQ ID NO: 44 - protein, 7 aa, Homo sapiens
DASNRAT

SEQ ID NO: 45 - protein, 9 aa, Homo sapiens
QQSINFPYT

SEQ ID NO: 46 - protein, 11 aa, Homo sapiens
RASQSISSWLA

SEQ ID NO: 47 - protein, 7 aa, Homo sapiens
KASSLES

SEQ ID NO: 48 - protein, 9 aa, Homo sapiens
QQYNSFSWT

SEQ ID NO: 49 - protein, 11 aa, Homo sapiens
RASQGISSWLA

SEQ ID NO: 50 - protein, 7 aa, Homo sapiens
AASSLQS

SEQ ID NO: 51 - protein, 9 aa, Homo sapiens
QQANSFPIT